European Patent Specification EP 3 145 943 B1, published March 13, 2024. Title: PEPTIDES, COMPOSITIONS COMPRISING THEM AND USES IN PARTICULAR COSMETIC USES. Applicant: SEDERMA. The sequence listing filed with the application follows.

SEQUENCE LISTING (23 sequences)

SEQ ID NO: 1 - protein, 5 aa, artificial sequence
  synthetic peptide
  MOD_RES (1)..(1): amidation by a Palmitoyl chain
KTTKS

SEQ ID NO: 2 - protein, 4 aa, artificial sequence
  synthetic peptide
  MOD_RES (1)..(1): amidation by a Palmitoyl chain
GQPR

SEQ ID NO: 3 - protein, 5 aa, Artificial sequence
  synthetic peptide
NIPPL

SEQ ID NO: 4 - protein, 4 aa, Artificial sequence
  synthetic peptide
IPPL

SEQ ID NO: 5 - protein, 4 aa, Artificial sequence
  synthetic peptide
VPPF

SEQ ID NO: 6 - protein, 6 aa, Artificial sequence
  synthetic peptide
PVVVPP

SEQ ID NO: 7 - protein, 4 aa, Artificial sequence
  synthetic peptide
FPPQ

SEQ ID NO: 8 - protein, 4 aa, Artificial organism
  synthetic peptide
LPPT

SEQ ID NO: 9 - protein, 4 aa, artificial sequence
  synthetic peptide
RSRK

SEQ ID NO: 10 - protein, 4 aa, artificial sequence
  synthetic peptide
GQPR

SEQ ID NO: 11 - protein, 4 aa, artificial sequence
  synthetic peptide
KTFK

SEQ ID NO: 12 - protein, 5 aa, artificial sequence
  synthetic peptide
KTTKS

SEQ ID NO: 13 - protein, 6 aa, artificial sequence
  Synthetic peptide
GKTTKS

SEQ ID NO: 14 - protein, 6 aa, artificial sequence
  synthetic peptide
VGVAPG

SEQ ID NO: 15 - protein, 4 aa, Artificial sequence
  Synthetic peptide
  MOD_RES (1)..(1): amidation by an Elaidoyl chain
KTFK

SEQ ID NO: 16 - protein, 5 aa, artificial sequence
  synthetic peptide
  MOD_RES (1)..(1): amidation by a Palmitoyl chain
  misc_feature (5)..(5): Xaa can be any naturally occurring amino acid
YGGFX

SEQ ID NO: 17 - protein, 6 aa, artificial sequence
  synthetic peptide
  MOD_RES (1)..(1): amidation by a Palmitoyl chain
VGVAPG

SEQ ID NO: 18 - protein, 6 aa, Artificial sequence
  Synthetic peptide
  MOD_RES (1)..(1): amidation by a Palmitoyl chain
GKTTKS

SEQ ID NO: 19 - protein, 6 aa, synthetic peptide
EEMQRR

SEQ ID NO: 20 - protein, 5 aa, synthetic peptide
YAGFL

SEQ ID NO: 21 - protein, 4 aa, synthetic peptide
AHSH

SEQ ID NO: 22 - protein, 6 aa, synthetic peptide
SIKVAV

SEQ ID NO: 23 - protein, 6 aa, synthetic peptide
GPQGPQ